European Patent Application EP 4 382 538 A1, published June 12, 2024. Title: anti-CD79b and anti-CD3 bispecific antibody and the use thereof. Applicant: INNOVENT BIOLOGICS (SUZHOU) CO., LTD. The sequence listing filed with the application follows.

SEQUENCE LISTING (72 sequences)

SEQ ID NO: 1 - protein, 10 aa, synthetic construct
GYTFTDYSMH

SEQ ID NO: 2 - protein, 17 aa, synthetic construct
WINTETGEPSYADDFKG

SEQ ID NO: 3 - skipped

SEQ ID NO: 4 - protein, 112 aa, synthetic construct
QVQLVQSGSELKKPGASVKVSCKASGYTFTDYSMHWVRQAPGQGLEWMGWINTETGEPSYADDFKGRFVFSLDTSVSTAYLQISSLKAEDTAVYYCYYGPYWGQGTLVTVSS

SEQ ID NO: 5 - protein, 442 aa, synthetic construct
QVQLVQSGSELKKPGASVKVSCKASGYTFTDYSMHWVRQAPGQGLEWMGWINTETGEPSYADDFKGRFVFSLDTSVSTAYLQISSLKAEDTAVYYCYYGPYWGQGTLVTVSSASTKGPSVFPLAPSSKSTSGGTAALGCLVKDYFPEPVTVSWNSGALTSGVHTFPAVLQSSGLYSLSSVVTVPSSSLGTQTYICNVNHKPSNTKVDKKVEPKSCDKTHTCPPCPAPEAAGGPSVFLFPPKPKDTLMISRTPEVTCVVVDVSHEDPEVKFNWYVDGVEVHNAKTKPREEQYNSTYRVVSVLTVLHQDWLNGKEYKCKVSNKALPAPIEKTISKAKGQPREPQVYTLPPSRDELTKNQVSLWCLVKGFYPSDIAVEWESNGQPENNYKTTPPVLDSDGSFFLYSKLTVDKSRWQQGNVFSCSVMHEALHNHYTQKSLSLSPGK

SEQ ID NO: 6 - protein, 15 aa, synthetic construct
KASQSVDHDVDSYMD

SEQ ID NO: 7 - protein, 7 aa, synthetic construct
SASNLES

SEQ ID NO: 8 - protein, 9 aa, synthetic construct
QQINEYPYT

SEQ ID NO: 9 - protein, 111 aa, synthetic construct
EIVLTQSPATLSLSPGERATLSCKASQSVDHDVDSYMDWYQQKPGQAPRLLIYSASNLESGIPARFSGSGSGTDFTLTISSLEPEDFAVYYCQQINEYPYTFGGGTKVEIK

SEQ ID NO: 10 - protein, 218 aa, synthetic construct
EIVLTQSPATLSLSPGERATLSCKASQSVDHDVDSYMDWYQQKPGQAPRLLIYSASNLESGIPARFSGSGSGTDFTLTISSLEPEDFAVYYCQQINEYPYTFGGGTKVEIKRTVAAPSVFIFPPSDEQLKSGTASVVCLLNNFYPREAKVQWKVDNALQSGNSQESVTEQDSKDSTYSLSSTLTLSKADYEKHKVYACEVTHQGLSSPVTKSFNRGEC

SEQ ID NO: 11 - protein, 10 aa, synthetic construct
GYTFTDYWVN

SEQ ID NO: 12 - protein, 17 aa, synthetic construct
MIDPSDSETHYNQMFND

SEQ ID NO: 13 - protein, 4 aa, synthetic construct
SNYY

SEQ ID NO: 14 - protein, 113 aa, synthetic construct
QVQLVQSGAEVKKPGASVKVSCKASGYTFTDYWVNWVRQAPGQGLEWMGMIDPSDSETHYNQMFNDRVTMTVDTSTSTVYMELSSLRSEDTAVYYCTRSNYYWGQGTLVTVSS

SEQ ID NO: 15 - protein, 443 aa, synthetic construct
QVQLVQSGAEVKKPGASVKVSCKASGYTFTDYWVNWVRQAPGQGLEWMGMIDPSDSETHYNQMFNDRVTMTVDTSTSTVYMELSSLRSEDTAVYYCTRSNYYWGQGTLVTVSSASTKGPSVFPLAPSSKSTSGGTAALGCLVKDYFPEPVTVSWNSGALTSGVHTFPAVLQSSGLYSLSSVVTVPSSSLGTQTYICNVNHKPSNTKVDKKVEPKSCDKTHTCPPCPAPEAAGGPSVFLFPPKPKDTLMISRTPEVTCVVVDVSHEDPEVKFNWYVDGVEVHNAKTKPREEQYNSTYRVVSVLTVLHQDWLNGKEYKCKVSNKALPAPIEKTISKAKGQPREPQVYTLPPSRDELTKNQVSLWCLVKGFYPSDIAVEWESNGQPENNYKTTPPVLDSDGSFFLYSKLTVDKSRWQQGNVFSCSVMHEALHNHYTQKSLSLSPGK

SEQ ID NO: 16 - protein, 16 aa, synthetic construct
KSSQSLLDSEGKTYLN

SEQ ID NO: 17 - protein, 7 aa, synthetic construct
LVSKLDS

SEQ ID NO: 18 - protein, 7 aa, synthetic construct
GTHFPLT

SEQ ID NO: 19 - protein, 112 aa, synthetic construct
DIVMTQTPLSLSVTPGQPASISCKSSQSLLDSEGKTYLNWLLQKPGQSPQSLIYLVSKLDSGVPDRFSGSGSGTDFTLKISRVEAEDVGVYYCWQGTHFPLTFGGGTKVEIK

SEQ ID NO: 20 - protein, 219 aa, synthetic construct
DIVMTQTPLSLSVTPGQPASISCKSSQSLLDSEGKTYLNWLLQKPGQSPQSLIYLVSKLDSGVPDRFSGSGSGTDFTLKISRVEAEDVGVYYCWQGTHFPLTFGGGTKVEIKRTVAAPSVFIFPPSDEQLKSGTASVVCLLNNFYPREAKVQWKVDNALQSGNSQESVTEQDSKDSTYSLSSTLTLSKADYEKHKVYACEVTHQGLSSPVTKSFNRGEC

SEQ ID NO: 21 - protein, 10 aa, synthetic construct
GYSFTTYWMN

SEQ ID NO: 22 - protein, 17 aa, synthetic construct
MIDPSDSETHYNHLFKD

SEQ ID NO: 23 - protein, 4 aa, synthetic construct
AIGY

SEQ ID NO: 24 - protein, 113 aa, synthetic construct
QVQLVQSGAEVKKPGASVKVSCKASGYSFTTYWMNWVRQAPGQGLTWMGMIDPSDSETHYNHLFKDRVTMTVDKSTSTAYMELSSLRSEDTAVYYCTRAIGYWGQGTLVTVSS

SEQ ID NO: 25 - protein, 443 aa, synthetic construct
QVQLVQSGAEVKKPGASVKVSCKASGYSFTTYWMNWVRQAPGQGLTWMGMIDPSDSETHYNHLFKDRVTMTVDKSTSTAYMELSSLRSEDTAVYYCTRAIGYWGQGTLVTVSSASTKGPSVFPLAPSSKSTSGGTAALGCLVKDYFPEPVTVSWNSGALTSGVHTFPAVLQSSGLYSLSSVVTVPSSSLGTQTYICNVNHKPSNTKVDKKVEPKSCDKTHTCPPCPAPEAAGGPSVFLFPPKPKDTLMISRTPEVTCVVVDVSHEDPEVKFNWYVDGVEVHNAKTKPREEQYNSTYRVVSVLTVLHQDWLNGKEYKCKVSNKALPAPIEKTISKAKGQPREPQVYTLPPSRDELTKNQVSLWCLVKGFYPSDIAVEWESNGQPENNYKTTPPVLDSDGSFFLYSKLTVDKSRWQQGNVFSCSVMHEALHNHYTQKSLSLSPGK

SEQ ID NO: 26 - protein, 16 aa, synthetic construct
KSSLSLLDSEGKTYLN

SEQ ID NO: 27 - protein, 7 aa, synthetic construct
LVSKLDS

SEQ ID NO: 28 - protein, 9 aa, synthetic construct
WQGTHFPLT

SEQ ID NO: 29 - protein, 112 aa, synthetic construct
DVVMTQSPLSLPVTLGQPASISCKSSLSLLDSEGKTYLNWFQQRPGQSPRPLISLVSKLDSGVPDRFSGSGSGTDFTLKISRVEAEDVGVYYCWQGTHFPLTFGGGTKVEIK

SEQ ID NO: 30 - protein, 219 aa, synthetic construct
DVVMTQSPLSLPVTLGQPASISCKSSLSLLDSEGKTYLNWFQQRPGQSPRPLISLVSKLDSGVPDRFSGSGSGTDFTLKISRVEAEDVGVYYCWQGTHFPLTFGGGTKVEIKRTVAAPSVFIFPPSDEQLKSGTASVVCLLNNFYPREAKVQWKVDNALQSGNSQESVTEQDSKDSTYSLSSTLTLSKADYEKHKVYACEVTHQGLSSPVTKSFNRGEC

SEQ ID NO: 31 - protein, 10 aa, synthetic construct
GFTFNTYAMN

SEQ ID NO: 32 - protein, 15 aa, synthetic construct
RIRSKYNNYATYYAD

SEQ ID NO: 33 - protein, 14 aa, synthetic construct
HYNFGQSYVSWFAY

SEQ ID NO: 34 - protein, 125 aa, synthetic construct
EVQLVESGGGLVQPGGSLKLSCAASGFTFNTYAMNWVRQASGKGLEWVGRIRSKYNNYATYYADSVKDRFTISRDDSKSTLYLQMNSLKTEDTAVYYCARHYNFGQSYVSWFAYWGQGTTVTVSS

SEQ ID NO: 35 - protein, 455 aa, synthetic construct
EVQLVESGGGLVQPGGSLKLSCAASGFTFNTYAMNWVRQASGKGLEWVGRIRSKYNNYATYYADSVKDRFTISRDDSKSTLYLQMNSLKTEDTAVYYCARHYNFGQSYVSWFAYWGQGTTVTVSSASTKGPSVFPLAPSSKSTSGGTAALGCLVKDYFPEPVTVSWNSGALTSGVHTFPAVLQSSGLYSLSSVVTVPSSSLGTQTYICNVNHKPSNTKVDKKVEPKSCDKTHTCPPCPAPEAAGGPSVFLFPPKPKDTLMISRTPEVTCVVVDVSHEDPEVKFNWYVDGVEVHNAKTKPREEQYNSTYRVVSVLTVLHQDWLNGKEYKCKVSNKALPAPIEKTISKAKGQPREPQVYTLPPSRDELTKNQVSLSCAVKGFYPSDIAVEWESNGQPENNYKTTPPVLDSDGSFFLVSKLTVDKSRWQQGNVFSCSVMHEALHNHYTQKSLSLSPGK

SEQ ID NO: 36 - protein, 14 aa, synthetic construct
RSSTGAVTTSNYAN

SEQ ID NO: 37 - protein, 7 aa, synthetic construct
GTNKRAP

SEQ ID NO: 38 - protein, 9 aa, synthetic construct
ALWYSNLWV

SEQ ID NO: 39 - protein, 109 aa, synthetic construct
QAVVTQEPSLTVSPGGTVTLTCRSSTGAVTTSNYANWVQQKPGQAPRGLIGGTNKRAPGVPARFSGSLLGDKAALTLLGAQPEDEAEYYCALWYSNLWVFGQGTKLTVL

SEQ ID NO: 40 - protein, 215 aa, synthetic construct
QAVVTQEPSLTVSPGGTVTLTCRSSTGAVTTSNYANWVQQKPGQAPRGLIGGTNKRAPGVPARFSGSLLGDKAALTLLGAQPEDEAEYYCALWYSNLWVFGQGTKLTVLGQPKAAPSVTLFPPSSEELQANKATLVCLISDFYPGAVTVAWKADSSPVKAGVETTTPSKQSNNKYAASSYLSLTPEQWKSHRSYSCQVTHEGSTVEKTVAPTECS

SEQ ID NO: 41 - protein, 10 aa, synthetic construct
GFTFNTYAMN

SEQ ID NO: 42 - protein, 19 aa, synthetic construct
RIRSKYNNYATYYADSVKD

SEQ ID NO: 43 - protein, 14 aa, synthetic construct
HGNFGQSYVSWFAY

SEQ ID NO: 44 - protein, 125 aa, synthetic construct
EVQLVESGGGLVQPGGSLKLSCAASGFTFNTYAMNWVRQASGKGLEWVGRIRSKYNNYATYYADSVKDRFTISRDDSKSTLYLQMNSLKTEDTAVYYCARHGNFGQSYVSWFAYWGQGTTVTVSS

SEQ ID NO: 45 - protein, 455 aa, synthetic construct
EVQLVESGGGLVQPGGSLKLSCAASGFTFNTYAMNWVRQASGKGLEWVGRIRSKYNNYATYYADSVKDRFTISRDDSKSTLYLQMNSLKTEDTAVYYCARHGNFGQSYVSWFAYWGQGTTVTVSSASTKGPSVFPLAPSSKSTSGGTAALGCLVKDYFPEPVTVSWNSGALTSGVHTFPAVLQSSGLYSLSSVVTVPSSSLGTQTYICNVNHKPSNTKVDKKVEPKSCDKTHTCPPCPAPEAAGGPSVFLFPPKPKDTLMISRTPEVTCVVVDVSHEDPEVKFNWYVDGVEVHNAKTKPREEQYNSTYRVVSVLTVLHQDWLNGKEYKCKVSNKALPAPIEKTISKAKGQPREPQVYTLPPSRDELTKNQVSLSCAVKGFYPSDIAVEWESNGQPENNYKTTPPVLDSDGSFFLVSKLTVDKSRWQQGNVFSCSVMHEALHNHYTQKSLSLSPGK

SEQ ID NO: 46 - protein, 14 aa, synthetic construct
RSSTGAVTTSNYAN

SEQ ID NO: 47 - protein, 7 aa, synthetic construct
GTNKRAP

SEQ ID NO: 48 - protein, 9 aa, synthetic construct
ALWYSNLWV

SEQ ID NO: 49 - protein, 109 aa, synthetic construct; identical to SEQ ID NO: 39

SEQ ID NO: 50 - protein, 215 aa, synthetic construct; identical to SEQ ID NO: 40

SEQ ID NO: 51 - protein, 10 aa, synthetic construct
GYTFTTYYMN

SEQ ID NO: 52 - protein, 17 aa, synthetic construct
MIDPSDSETHYNQKFQG

SEQ ID NO: 53 - protein, 4 aa, synthetic construct
SLAF

SEQ ID NO: 54 - protein, 113 aa, synthetic construct
EVQLVQSGAEVKKPGASVKVSCKASGYTFTTYYMNWVRQAPGQGLEWIGMIDPSDSETHYNQKFQGRATLTVDTSTSTAYLELSSLRSEDTAVYYCSRSLAFWGQGTLVTVSS

SEQ ID NO: 55 - protein, 443 aa, synthetic construct
EVQLVQSGAEVKKPGASVKVSCKASGYTFTTYYMNWVRQAPGQGLEWIGMIDPSDSETHYNQKFQGRATLTVDTSTSTAYLELSSLRSEDTAVYYCSRSLAFWGQGTLVTVSSASTKGPSVFPLAPSSKSTSGGTAALGCLVKDYFPEPVTVSWNSGALTSGVHTFPAVLQSSGLYSLSSVVTVPSSSLGTQTYICNVNHKPSNTKVDKKVEPKSCDKTHTCPPCPAPEAAGGPSVFLFPPKPKDTLMISRTPEVTCVVVDVSHEDPEVKFNWYVDGVEVHNAKTKPREEQYNSTYRVVSVLTVLHQDWLNGKEYKCKVSNKALPAPIEKTISKAKGQPREPQVYTLPPSRDELTKNQVSLWCLVKGFYPSDIAVEWESNGQPENNYKTTPPVLDSDGSFFLYSKLTVDKSRWQQGNVFSCSVMHEALHNHYTQKSLSLSPGK

SEQ ID NO: 56 - protein, 16 aa, synthetic construct
KSSQSLLDSDGKTYLN

SEQ ID NO: 57 - protein, 7 aa, synthetic construct
LVSKLDS

SEQ ID NO: 58 - protein, 9 aa, synthetic construct
WQGTHFPQT

SEQ ID NO: 59 - protein, 112 aa, synthetic construct
DIVMTQTPLSLPVTPGQPASISCKSSQSLLDSDGKTYLNWLLQKPGQSPQSLIYLVSKLDSGVPDRFSGSGSGTDFTLKISRVEAEDVGVYYCWQGTHFPQTFGQGTKVEIK

SEQ ID NO: 60 - protein, 219 aa, synthetic construct
DIVMTQTPLSLPVTPGQPASISCKSSQSLLDSDGKTYLNWLLQKPGQSPQSLIYLVSKLDSGVPDRFSGSGSGTDFTLKISRVEAEDVGVYYCWQGTHFPQTFGQGTKVEIKRTVAAPSVFIFPPSDEQLKSGTASVVCLLNNFYPREAKVQWKVDNALQSGNSQESVTEQDSKDSTYSLSSTLTLSKADYEKHKVYACEVTHQGLSSPVTKSFNRGEC

SEQ ID NO: 61 - protein, 10 aa, synthetic construct
GFTFTSYYIH

SEQ ID NO: 62 - protein, 17 aa, synthetic construct
WIYPENDNTKYNEKFKD

SEQ ID NO: 63 - protein, 10 aa, synthetic construct
DGYSRYYFDY

SEQ ID NO: 64 - protein, 119 aa, synthetic construct
EVQLVQSGAEVKKPGASVKVSCKASGFTFTSYYIHWVRQAPGQGLEWIGWIYPENDNTKYNEKFKDRVTITADTSTSTAYLELSSLRSEDTAVYYCARDGYSRYYFDYWGQGTLVTVSS

SEQ ID NO: 65 - protein, 449 aa, synthetic construct
EVQLVQSGAEVKKPGASVKVSCKASGFTFTSYYIHWVRQAPGQGLEWIGWIYPENDNTKYNEKFKDRVTITADTSTSTAYLELSSLRSEDTAVYYCARDGYSRYYFDYWGQGTLVTVSSASTKGPSVFPLAPSSKSTSGGTAALGCLVKDYFPEPVTVSWNSGALTSGVHTFPAVLQSSGLYSLSSVVTVPSSSLGTQTYICNVNHKPSNTKVDKKVEPKSCDKTHTCPPCPAPEAAGGPSVFLFPPKPKDTLMISRTPEVTCVVVDVSHEDPEVKFNWYVDGVEVHNAKTKPREEQYNSTYRVVSVLTVLHQDWLNGKEYKCKVSNKALPAPIEKTISKAKGQPREPQVYTLPPSRDELTKNQVSLSCAVKGFYPSDIAVEWESNGQPENNYKTTPPVLDSDGSFFLVSKLTVDKSRWQQGNVFSCSVMHEALHNHYTQKSLSLSPGK

SEQ ID NO: 66 - protein, 17 aa, synthetic construct
KSSQSLLNSRTRKNYLA

SEQ ID NO: 67 - protein, 7 aa, synthetic construct
WTSTRKS

SEQ ID NO: 68 - protein, 8 aa, synthetic construct
KQSFILRT

SEQ ID NO: 69 - protein, 112 aa, synthetic construct
DIVMTQSPDSLAVSLGERATINCKSSQSLLNSRTRKNYLAWYQQKPGQSPKLLIYWTSTRKSGVPDRFSGSGSGTDFTLTISSLQAEDVAVYYCKQSFILRTFGQGTKVEIK

SEQ ID NO: 70 - protein, 219 aa, synthetic construct
DIVMTQSPDSLAVSLGERATINCKSSQSLLNSRTRKNYLAWYQQKPGQSPKLLIYWTSTRKSGVPDRFSGSGSGTDFTLTISSLQAEDVAVYYCKQSFILRTFGQGTKVEIKRTVAAPSVFIFPPSDEQLKSGTASVVCLLNNFYPREAKVQWKVDNALQSGNSQESVTEQDSKDSTYSLSSTLTLSKADYEKHKVYACEVTHQGLSSPVTKSFNRGEC

SEQ ID NO: 71 - protein, 447 aa, synthetic construct
EVQLVESGGGLVQPGGSLRLSCAASGYTFSSYWIEWVRQAPGKGLEWIGEILPGGGDTNYNEIFKGRATFSADTSKNTAYLQMNSLRAEDTAVYYCTRRVPIRLDYWGQGTLVTVSSASTKGPSVFPLAPSSKSTSGGTAALGCLVKDYFPEPVTVSWNSGALTSGVHTFPAVLQSSGLYSLSSVVTVPSSSLGTQTYICNVNHKPSNTKVDKKVEPKSCDKTHTCPPCPAPELLGGPSVFLFPPKPKDTLMISRTPEVTCVVVDVSHEDPEVKFNWYVDGVEVHNAKTKPREEQYNSTYRVVSVLTVLHQDWLNGKEYKCKVSNKALPAPIEKTISKAKGQPREPQVYTLPPSRDELTKNQVSLTCLVKGFYPSDIAVEWESNGQPENNYKTTPPVLDSDGSFFLYSKLTVDKSRWQQGNVFSCSVMHEALHNHYTQKSLSLSPGK

SEQ ID NO: 72 - protein, 218 aa, synthetic construct
DIQLTQSPSSLSASVGDRVTITCKASQSVDYEGDSFLNWYQQKPGKAPKLLIYAASNLESGVPSRFSGSGSGTDFTLTISSLQPEDFATYYCQQSNEDPLTFGQGTKVEIKRTVAAPSVFIFPPSDEQLKSGTASVVCLLNNFYPREAKVQWKVDNALQSGNSQESVTEQDSKDSTYSLSSTLTLSKADYEKHKVYACEVTHQGLSSPVTKSFNRGEC